European Patent Specification EP 4 098 247 B1, published August 20, 2025. Title: Stabilized Formulations Containing Anti-Interleukin-6 Receptor (IL-6R) Antibodies. Applicant: Dix, Daniel Walsh, Scott Graham, Kenneth Kamen, Douglas. Application To be assigned. The sequence listing filed with the application follows.

SEQUENCE LISTING (74 sequences)

SEQ ID NO: 1 - DNA, 379 bp, Artificial Sequence
  Synthetic
gaagtgcagctggtggagtctgggggaaacttggtacagcctggcaggtccctgagactctcctgtgcagcctctggattcatctttgatgattatgccatgcactgggtccggcaagctccagggaagggcctggagtgggtctcaggtattagttggaatagtggtagcataggctatgcggactctgtgaagggccgattcaccatctccagagacaacgccaagaactccctgtatctgcaaatgaacagtctgagagctgaggacacggccttgtattactgtgcaaaagatggaggcagcagctggttaccgttcgtctactactacggtatggacgtctggggccaagggaccacggtcaccgtctcgtcag

SEQ ID NO: 2 - protein, 126 aa, Artificial Sequence
  Synthetic
EVQLVESGGNLVQPGRSLRLSCAASGFIFDDYAMHWVRQAPGKGLEWVSGISWNSGSIGYADSVKGRFTISRDNAKNSLYLQMNSLRAEDTALYYCAKDGGSSWLPFVYYYGMDVWGQGTTVTVSS

SEQ ID NO: 3 - DNA, 24 bp, Artificial Sequence
  Synthetic
ggattcatctttgatgattatgcc

SEQ ID NO: 4 - protein, 8 aa, Artificial Sequence
  Synthetic
GFIFDDYA

SEQ ID NO: 5 - DNA, 24 bp, Artificial Sequence
  Synthetic
attagttggaatagtggtagcata

SEQ ID NO: 6 - protein, 8 aa, Artificial Sequence
  Synthetic
ISWNSGSI

SEQ ID NO: 7 - DNA, 57 bp, Artificial Sequence
  Synthetic
gcaaaagatggaggcagcagctggttaccgttcgtctactactacggtatggacgtc

SEQ ID NO: 8 - protein, 19 aa, Artificial Sequence
  Synthetic
AKDGGSSWLPFVYYYGMDV

SEQ ID NO: 9 - DNA, 325 bp, Artificial Sequence
  Synthetic
gaaatagtgatgacgcagtctccagccaccctgtctgtgtctcccggggaaagagccaccctctcctgcagggccagtcagagtattagcagcaactttgcctggtaccagcagaaacctggccaggctcccaggctcctcatctatggtgcatccaccagggccactggtatcccagccaggttcagtggcagtgggtctgggacagacttcactctcaccatcagcagcctgcagtctgaagattttgcagtttattactgtcagcagtatagtagctggcctccgtacacttttggccaggggaccaagctggagatcaaac

SEQ ID NO: 10 - protein, 108 aa, Artificial Sequence
  Synthetic
EIVMTQSPATLSVSPGERATLSCRASQSISSNFAWYQQKPGQAPRLLIYGASTRATGIPARFSGSGSGTDFTLTISSLQSEDFAVYYCQQYSSWPPYTFGQGTKLEIK

SEQ ID NO: 11 - DNA, 18 bp, Artificial Sequence
  Synthetic
cagagtattagcagcaac

SEQ ID NO: 12 - protein, 6 aa, Artificial Sequence
  Synthetic
QSISSN

SEQ ID NO: 13 - DNA, 9 bp, Artificial Sequence
  Synthetic
ggtgcatcc

SEQ ID NO: 14 - protein, 3 aa, Artificial Sequence
  Synthetic
GAS

SEQ ID NO: 15 - DNA, 30 bp, Artificial Sequence
  Synthetic
cagcagtatagtagctggcctccgtacact

SEQ ID NO: 16 - protein, 10 aa, Artificial Sequence
  Synthetic
QQYSSWPPYT

SEQ ID NO: 17 - DNA, 349 bp, Artificial Sequence
  Synthetic
gaagtgcagctggtggagtctgggggaggcttggttcagcctggcaggtccctgagactctcctgtgcagcctctagatttacctttgatgattatgccatgcactgggtccggcaagctccagggaagggcctggagtgggtctcaggtattagttggaatagtggtagaataggttatgcggactctgtgaagggccgattcaccatctccagagacaacgccgagaactccctctttctgcaaatgaacggtctgagagcagaggacacggccttgtattactgtgcaaaaggccgagattcttttgatatctggggccaagggacaatggtcaccgtctcttcag

SEQ ID NO: 18 - protein, 116 aa, Artificial Sequence
  Synthetic
EVQLVESGGGLVQPGRSLRLSCAASRFTFDDYAMHWVRQAPGKGLEWVSGISWNSGRIGYADSVKGRFTISRDNAENSLFLQMNGLRAEDTALYYCAKGRDSFDIWGQGTMVTVSS

SEQ ID NO: 19 - DNA, 24 bp, Artificial Sequence
  Synthetic
agatttacctttgatgattatgcc

SEQ ID NO: 20 - protein, 8 aa, Artificial Sequence
  Synthetic
RFTFDDYA

SEQ ID NO: 21 - DNA, 24 bp, Artificial Sequence
  Synthetic
attagttggaatagtggtagaata

SEQ ID NO: 22 - protein, 8 aa, Artificial Sequence
  Synthetic
ISWNSGRI

SEQ ID NO: 23 - DNA, 27 bp, Artificial Sequence
  Synthetic
gcaaaaggccgagattcttttgatatc

SEQ ID NO: 24 - protein, 9 aa, Artificial Sequence
  Synthetic
AKGRDSFDI

SEQ ID NO: 25 - DNA, 322 bp, Artificial Sequence
  Synthetic
gacatccagatgacccagtctccatcttccgtgtctgcatctgtaggagacagagtcaccatcacttgtcgggcgagtcagggtattagcagctggttagcctggtatcagcagaaaccagggaaagcccctaagctcctgatctatggtgcatccagtttggaaagtggggtcccatcaaggttcagcggcagtggatctgggacagatttcactctcaccatcagcagcctgcagcctgaagattttgcaagttattattgtcaacaggctaacagtttcccgtacacttttggccaggggaccaagctggagatcaaac

SEQ ID NO: 26 - protein, 107 aa, Artificial Sequence
  Synthetic
DIQMTQSPSSVSASVGDRVTITCRASQGISSWLAWYQQKPGKAPKLLIYGASSLESGVPSRFSGSGSGTDFTLTISSLQPEDFASYYCQQANSFPYTFGQGTKLEIK

SEQ ID NO: 27 - DNA, 18 bp, Artificial Sequence
  Synthetic
cagggtattagcagctgg

SEQ ID NO: 28 - protein, 6 aa, Artificial Sequence
  Synthetic
QGISSW

SEQ ID NO: 29 - DNA, 9 bp, Artificial Sequence
  Synthetic
ggtgcatcc

SEQ ID NO: 30 - protein, 3 aa, Artificial Sequence
  Synthetic
GAS

SEQ ID NO: 31 - DNA, 27 bp, Artificial Sequence
  Synthetic
caacaggctaacagtttcccgtacact

SEQ ID NO: 32 - protein, 9 aa, Artificial Sequence
  Synthetic
QQANSFPYT

SEQ ID NO: 33 - DNA, 349 bp, Artificial Sequence
  Synthetic
gaagtgcagctggtggagtctgggggaggcttggtacagcctggcaggtccctgagactctcctgtgcagcctctggattcacctttgatgattatgccctgcactgggtccggcaagctccagggaagggcctggagtgggtctcaggtgttagttggaatggtggtagaataggctatgcggactctgtgaaaggccgattcaccatctccagagacaacgccaagaactccctctttctgcaaatgaacagtctgagagttgaggacacggccttgtattattgtgcaaaaggccgggatgcttttgatatctggggccaagggacattggtcaccgtctcttcag

SEQ ID NO: 34 - protein, 116 aa, Artificial Sequence
  Synthetic
EVQLVESGGGLVQPGRSLRLSCAASGFTFDDYALHWVRQAPGKGLEWVSGVSWNGGRIGYADSVKGRFTISRDNAKNSLFLQMNSLRVEDTALYYCAKGRDAFDIWGQGTLVTVSS

SEQ ID NO: 35 - DNA, 24 bp, Artificial Sequence
  Synthetic
ggattcacctttgatgattatgcc

SEQ ID NO: 36 - protein, 8 aa, Artificial Sequence
  Synthetic
GFTFDDYA

SEQ ID NO: 37 - DNA, 24 bp, Artificial Sequence
  Synthetic
gttagttggaatggtggtagaata

SEQ ID NO: 38 - protein, 8 aa, Artificial Sequence
  Synthetic
VSWNGGRI

SEQ ID NO: 39 - DNA, 27 bp, Artificial Sequence
  Synthetic
gcaaaaggccgggatgcttttgatatc

SEQ ID NO: 40 - protein, 9 aa, Artificial Sequence
  Synthetic
AKGRDAFDI

SEQ ID NO: 41 - DNA, 322 bp, Artificial Sequence
  Synthetic
gacatccagatgacccagtctccatcttccgtgtctgcatctgtaggagacagagtcaccatcacttgtcgggcgagtcagggtattagcagctggttagcctggtatcagcagaaaccagggaaagcccctaaactcctgatctatgctgcatccagtttgcaaagtggggtcccatcaaggttcagcggcagtggatctgggacagatttcactctcaccatcagcagcctgcagcctgaagattttgcaacttactattgtcaacatgcttacagtttcccgtacacttttggccaggggaccaagctggagatcaaac

SEQ ID NO: 42 - protein, 107 aa, Artificial Sequence
  Synthetic
DIQMTQSPSSVSASVGDRVTITCRASQGISSWLAWYQQKPGKAPKLLIYAASSLQSGVPSRFSGSGSGTDFTLTISSLQPEDFATYYCQHAYSFPYTFGQGTKLEIK

SEQ ID NO: 43 - DNA, 18 bp, Artificial Sequence
  Synthetic
cagggtattagcagctgg

SEQ ID NO: 44 - protein, 6 aa, Artificial Sequence
  Synthetic
QGISSW

SEQ ID NO: 45 - DNA, 9 bp, Artificial Sequence
  Synthetic
gctgcatcc

SEQ ID NO: 46 - protein, 3 aa, Artificial Sequence
  Synthetic
AAS

SEQ ID NO: 47 - DNA, 27 bp, Artificial Sequence
  Synthetic
caacatgcttacagtttcccgtacact

SEQ ID NO: 48 - protein, 9 aa, Artificial Sequence
  Synthetic
QHAYSFPYT

SEQ ID NO: 49 - DNA, 361 bp, Artificial Sequence
  Synthetic
caggtgcagctggtgcagtctggggctgaggtgaaagagcctggggcctcagtgaaggtctcctgcaaggcttctggatacaccttcacctcttatgatatcatctgggtgcgacaggccactggacaagggcttgagtggatgggatggatgaacccaaacagtggtaacacaggctatacacagaacctccagggcagagtcaccttgaccaggaacacctccataactacagtctacatggaactgagcagcctgagctctgaggacacggccgtttattactgtgcgcgagactacagtagccactactacggtttggacgtctggggccaagggaccacggtcaccgtctcctcaa

SEQ ID NO: 50 - protein, 120 aa, Artificial Sequence
  Synthetic
QVQLVQSGAEVKEPGASVKVSCKASGYTFTSYDIIWVRQATGQGLEWMGWMNPNSGNTGYTQNLQGRVTLTRNTSITTVYMELSSLSSEDTAVYYCARDYSSHYYGLDVWGQGTTVTVSS

SEQ ID NO: 51 - DNA, 24 bp, Artificial Sequence
  Synthetic
ggatacaccttcacctcttatgat

SEQ ID NO: 52 - protein, 8 aa, Artificial Sequence
  Synthetic
GYTFTSYD

SEQ ID NO: 53 - DNA, 24 bp, Artificial Sequence
  Synthetic
atgaacccaaacagtggtaacaca

SEQ ID NO: 54 - protein, 8 aa, Artificial Sequence
  Synthetic
MNPNSGNT

SEQ ID NO: 55 - DNA, 39 bp, Artificial Sequence
  Synthetic
gcgcgagactacagtagccactactacggtttggacgtc

SEQ ID NO: 56 - protein, 13 aa, Artificial Sequence
  Synthetic
ARDYSSHYYGLDV

SEQ ID NO: 57 - DNA, 322 bp, Artificial Sequence
  Synthetic
gacatccagttgacccagtctccatccttcctgtctacatctataggagacagagtcaccatcacttgctgggccagtcaggacattagcaattatttagcctggtatcagcaaaaaccagggaaagcccctaagctcctgatctttgttgcatccactttgcagagtggggtcccatcaaggttcagcggcagtggatctgggacagaattcactctcacaatcagtagcctgcagcctgaggattttgcaacttattactgtcaacagtttaatagttacccgctcactttcggcggagggaccaaggtggaaatcaaac

SEQ ID NO: 58 - protein, 107 aa, Artificial Sequence
  Synthetic
DIQLTQSPSFLSTSIGDRVTITCWASQDISNYLAWYQQKPGKAPKLLIFVASTLQSGVPSRFSGSGSGTEFTLTISSLQPEDFATYYCQQFNSYPLTFGGGTKVEIK

SEQ ID NO: 59 - DNA, 18 bp, Artificial Sequence
  Synthetic
caggacattagcaattat

SEQ ID NO: 60 - protein, 6 aa, Artificial Sequence
  Synthetic
QDISNY

SEQ ID NO: 61 - DNA, 9 bp, Artificial Sequence
  Synthetic
gttgcatcc

SEQ ID NO: 62 - protein, 3 aa, Artificial Sequence
  Synthetic
VAS

SEQ ID NO: 63 - DNA, 30 bp, Artificial Sequence
  Synthetic
caacagtttaatagttacccgctcactttc

SEQ ID NO: 64 - protein, 10 aa, Artificial Sequence
  Synthetic
QQFNSYPLTF

SEQ ID NO: 65 - protein, 8 aa, Artificial Sequence
  Synthetic
  VARIANT (1)...(1): Xaa = Gly or Arg
  VARIANT (2)...(2): Xaa = Phe or Tyr
  VARIANT (3)...(3): Xaa = Ile or Thr
  VARIANT (4)...(4): Xaa = Phe
  VARIANT (5)...(5): Xaa = Asp or Thr
  VARIANT (6)...(6): Xaa = Asp or Ser
  VARIANT (7)...(7): Xaa = Tyr
  VARIANT (8)...(8): Xaa = Ala or Asp
XXXXXXXX

SEQ ID NO: 66 - protein, 8 aa, Artificial Sequence
  Synthetic
  VARIANT (1)...(1): Xaa = Ile, Val or Met
  VARIANT (2)...(2): Xaa = Ser or Asn
  VARIANT (3)...(3): Xaa = Thr or Pro
  VARIANT (4)...(4): Xaa = Asn
  VARIANT (5)...(5): Xaa = Ser or Gly
  VARIANT (6)...(6): Xaa = Gly
  VARIANT (7)...(7): Xaa = Ser, Arg or Asn
  VARIANT (8)...(8): Xaa = Ile or Thr
XXXXXXXX

SEQ ID NO: 67 - protein, 19 aa, Artificial Sequence
  Synthetic
  VARIANT (1)...(1): Xaa = Ala
  VARIANT (2)...(2): Xaa = Lys or Arg
  VARIANT (3)...(3): Xaa = Asp or Gly
  VARIANT (4)...(4): Xaa = Gly, Arg or Tyr
  VARIANT (5)...(5): Xaa = Gly, Asp or Ser
  VARIANT (6)...(6): Xaa = Ser or Ala
  VARIANT (7)...(7): Xaa = Ser, Phe or His
  VARIANT (8)...(8): Xaa = Trp, Asp or Tyr
  VARIANT (9)...(9): Xaa = Leu, Ile or Tyr
  VARIANT (10)...(10): Xaa = Pro, Gly or absent
  VARIANT (11)...(11): Xaa = Phe, Leu or absent
  VARIANT (12)...(12): Xaa = Val, Asp or absent
  VARIANT (13)...(13): Xaa = Tyr, Val or absent
  VARIANT (14)...(14): Xaa = Tyr or absent
  VARIANT (15)...(15): Xaa = Tyr or absent
  VARIANT (16)...(16): Xaa = Gly or absent
  VARIANT (17)...(17): Xaa = Met or absent
  VARIANT (18)...(18): Xaa = Asp or absent
  VARIANT (19)...(19): Xaa = Val or absent
XXXXXXXXXXXXXXXXXXX

SEQ ID NO: 68 - protein, 6 aa, Artificial Sequence
  Synthetic
  VARIANT (1)...(1): Xaa = Gln
  VARIANT (2)...(2): Xaa = Ser, Gly or Asp
  VARIANT (3)...(3): Xaa = Ile
  VARIANT (4)...(4): Xaa = Ser
  VARIANT (5)...(5): Xaa = Ser or Asn
  VARIANT (6)...(6): Xaa = Asn, Trp or Tyr
XXXXXX

SEQ ID NO: 69 - protein, 3 aa, Artificial Sequence
  Synthetic
  VARIANT (1)...(1): Xaa = Gly, Ala or Val
  VARIANT (2)...(2): Xaa = Ala
  VARIANT (3)...(3): Xaa = Ser
XXX

SEQ ID NO: 70 - protein, 10 aa, Artificial Sequence
  Synthetic
  VARIANT (1)...(1): Xaa = Gln
  VARIANT (2)...(2): Xaa = Gln or His
  VARIANT (3)...(3): Xaa = Tyr, Ala or Phe
  VARIANT (4)...(4): Xaa = Ser, Asn or Tyr
  VARIANT (5)...(5): Xaa = Ser
  VARIANT (6)...(6): Xaa = Trp, Phe or Tyr
  VARIANT (7)...(7): Xaa = Pro
  VARIANT (8)...(8): Xaa = Pro, Tyr or Leu
  VARIANT (9)...(9): Xaa = Tyr or Thr
  VARIANT (10)...(10): Xaa = Thr or absent
XXXXXXXXXX

SEQ ID NO: 71 - protein, 330 aa, Artificial Sequence [sequence omitted]

SEQ ID NO: 72 - protein, 327 aa, Artificial Sequence
  Synthetic
ASTKGPSVFPLAPCSRSTSESTAALGCLVKDYFPEPVTVSWNSGALTSGVHTFPAVLQSSGLYSLSSVVTVPSSSLGTKTYTCNVDHKPSNTKVDKRVESKYGPPCPSCPAPEFLGGPSVFLFPPKPKDTLMISRTPEVTCVVVDVSQEDPEVQFNWYVDGVEVHNAKTKPREEQFNSTYRVVSVLTVLHQDWLNGKEYKCKVSNKGLPSSIEKTISKAKGQPREPQVYTLPPSQEEMTKNQVSLTCLVKGFYPSDIAVEWESNGQPENNYKTTPPVLDSDGSFFLYSRLTVDKSRWQEGNVFSCSVMHEALHNHYTQKSLSLSLGK

SEQ ID NO: 73 - protein, 327 aa, Artificial Sequence
  Synthetic
ASTKGPSVFPLAPCSRSTSESTAALGCLVKDYFPEPVTVSWNSGALTSGVHTFPAVLQSSGLYSLSSVVTVPSSSLGTKTYTCNVDHKPSNTKVDKRVESKYGPPCPPCPAPEFLGGPSVFLFPPKPKDTLMISRTPEVTCVVVDVSQEDPEVQFNWYVDGVEVHNAKTKPREEQFNSTYRVVSVLTVLHQDWLNGKEYKCKVSNKGLPSSIEKTISKAKGQPREPQVYTLPPSQEEMTKNQVSLTCLVKGFYPSDIAVEWESNGQPENNYKTTPPVLDSDGSFFLYSRLTVDKSRWQEGNVFSCSVMHEALHNHYTQKSLSLSLGK

SEQ ID NO: 74 - protein, 358 aa, Homo sapiens
MVAVGCALLAALLAAPGAALAPRRCPAQEVARGVLTSLPGDSVTLTCPGVEPEDNATVHWVLRKPAAGSHPSRWAGMGRRLLLRSVQLHDSGNYSCYRAGRPAGTVHLLVDVPPEEPQLSCFRKSPLSNVVCEWGPRSTPSLTTKAVLLVRKFQNSPAEDFQEPCQYSQESQKFSCQLAVPEGDSSFYIVSMCVASSVGSKFSKTQTFQGCGILQPDPPANITVTAVARNPRWLSVTWQDPHSWNSSFYRLRFELRYRAERSKTFTTWMVKDLQHHCVIHDAWSGLRHVVQLRAQEEFGQGEWSEWSPEAMGTPWTESRSPPAENEVSTPMQALTTNKDDDNILFRDSANATSLPVQD